European Patent Application EP 4 162 946 A1, published April 12, 2023. Title: KYNURENINE AMINOTRANSFERASE AND PRODUCTS THEREOF FOR THE TREATMENT OF INFLAMMATORY BOWEL DISEASES. Applicant: Institut national de recherche pour l'agriculture, l'alimentation et l'environnement Institut des sciences et industries du vivant et de l'environnement Sorbonne Université Institut national de la santé et de la recherche médicale ASSISTANCE PUBLIQUE - HOPITAUX DE PARIS. The sequence listing filed with the application follows.

SEQUENCE LISTING (32 sequences)

SEQ ID NO: 1 - protein, 422 aa, Homo sapiens
MAKQLQARRLDGIDYNPWVEFVKLASEHDVVNLGQGFPDFPPPDFAVEAFQHAVSGDFMLNQYTKTFGYPPLTKILASFFGELLGQEIDPLRNVLVTVGGYGALFTAFQALVDEGDEVIIIEPFFDCYEPMTMMAGGRPVFVSLKPGPIQNGELGSSSNWQLDPMELAGKFTSRTKALVLNTPNNPLGKVFSREELELVASLCQQHDVVCITDEVYQWMVYDGHQHISIASLPGMWERTLTIGSAGKTFSATGWKVGWVLGPDHIMKHLRTVHQNSVFHCPTQSQAAVAESFEREQLLFRQPSSYFVQFPQAMQRCRDHMIRSLQSVGLKPIIPQGSYFLITDISDFKRKMPDLPGAVDEPYDRRFVKWMIKNKGLVAIPVSIFYSVPHQKHFDHYIRFCFVKDEATLQAMDEKLRKWKVEL

SEQ ID NO: 2 - protein, 372 aa, Homo sapiens
MAKQLQARRLDGIDYNPWVEFVKLASEHDVVNLGQGFPDFPPPDFAVEAFQHAVSGDFMLNQYTKTFVIIIEPFFDCYEPMTMMAGGRPVFVSLKPGPIQNGELGSSSNWQLDPMELAGKFTSRTKALVLNTPNNPLGKVFSREELELVASLCQQHDVVCITDEVYQWMVYDGHQHISIASLPGMWERTLTIGSAGKTFSATGWKVGWVLGPDHIMKHLRTVHQNSVFHCPTQSQAAVAESFEREQLLFRQPSSYFVQFPQAMQRCRDHMIRSLQSVGLKPIIPQGSYFLITDISDFKRKMPDLPGAVDEPYDRRFVKWMIKNKGLVAIPVSIFYSVPHQKHFDHYIRFCFVKDEATLQAMDEKLRKWKVEL

SEQ ID NO: 3 - protein, 250 aa, Homo sapiens
MAKQLQARRLDGIDYNPWVEFVKLASEHDVVNLGQGFPDFPPPDFAVEAFQHAVSGDFMLNQYTKTFGYPPLTKILASFFGELLGQEIDPLRNVLVTVGGYGALFTAFQALVDEGDEVIIIEPFFDCYEPMTMMAGGRPVFVSLKPGPIQNGELGSSSNWQLDPMELAGKFTSRTKALVLNTPNNPLGKVFSREELELVASLCQQHDVVCITDEVYQWMVYDGHQHISIVSAAVLFGLGQPASLACGNGP

SEQ ID NO: 4 - protein, 457 aa, Rattus norvegicus
MFRSAAALSVHLMWPLWGRKAGASLTRCLHQSLTMTKRLQARRLDGIDQNLWVEFGKLTKEYDVVNLGQGFPDFSPPDFATQAFQQATSGNFMLNQYTRAFGYPPLTNVLASFFGKLLGQEMDPLTNVLVTVGAYGALFTRFQALVDEGDEVIIMEPAFDCYEPMTMMAGGCPVFVTLKPSPAPKGKLGASNDWQLDPAELASKFTPRTKILVLNTPNNPLGKVFSRMELELVANLCQQHDVVCISDEVYQWLVYDGHQHVSIASLPGMWDRTLTIGSAGKSFSATGWKVGWVMGPDNIMKHLRTVHQNSIFHCPTQAQAAVAQCFEREQQHFGQPSSYFLQLPQAMELNRDHMIRSLQSVGLKLWISQGSYFLIADISDFKSKMPDLPGAEDEPYDRRFAKWMIKNMGLVGIPVSTFFSRPHQKDFDHYIRFCFVKDKATLQAMDERLRKWKELQP

SEQ ID NO: 5 - protein, 423 aa, Rattus norvegicus
MTKRLQARRLDGIDQNLWVEFGKLTKEYDVVNLGQGFPDFSPPDFATQAFQQATSGNFMLNQYTRAFGYPPLTNVLASFFGKLLGQEMDPLTNVLVTVGAYGALFTRFQALVDEGDEVIIMEPAFDCYEPMTMMAGGCPVFVTLKPSPAPKGKLGASNDWQLDPAELASKFTPRTKILVLNTPNNPLGKVFSRMELELVANLCQQHDVVCISDEVYQWLVYDGHQHVSIASLPGMWDRTLTIGSAGKSFSATGWKVGWVMGPDNIMKHLRTVHQNSIFHCPTQAQAAVAQCFEREQQHFGQPSSYFLQLPQAMELNRDHMIRSLQSVGLKLWISQGSYFLIADISDFKSKMPDLPGAEDEPYDRRFAKWMIKNMGLVGIPVSTFFSRPHQKDFDHYIRFCFVKDKATLQAMDERLRKWKELQP

SEQ ID NO: 6 - protein, 424 aa, Mus musculus
MSKQLQARRLEGIDHNPWVEFTRLSKEYDVVNLGQGFPDFSPPDFAVQAFQQATTGNFMLNQYTSAFGYPPLTKILASFFGKLLGQEMDPLKNVLVTVGAYGALFTAFQALVDEGDEVIIIEPAFNCYEPMTMMAGGRPVFVSLRLSPAPKGQLGSSNDWQLDPTELASKFTPRTKILVLNTPNNPLGKVFSKKELELVAALCQQHDVLCFSDEVYQWLVYDGHQHISIASLPGMWERTLTIGSAGKSFSATGWKVGWVMGPDNIMKHLRTVHQNSIFHCPTQAQAAVAQCFEREQQHFGQPSSYFLQLPQAMGLNRDHMIQSLQSVGLKPLIPQGSYFLIADISDFKSSMPDLPGAMDEPYDTRFAKWMIKNKGLSAIPVSTFYSQPHHKDFDHYIRFCFVKDKATLQAMDKRLCSWKGEPQA

SEQ ID NO: 7 - protein, 422 aa, Pan troglodytes
MAKQLQARRLDGIDYNPWVEFVKLASEHDVVNLGQGFPDFPPPEFAVEAFQHAVSGDFMLNQYTKTFGYPPLTKILASFFGKLLGQEIDPLRNVLVTVGGYGALFTAFQALVDEGDEVIIIEPFFDCYEPMTMMAGGHPVFVPLKPGPIQNGELGSSSNWQLDPMELASKFTSRTKALVLNTPNNPLGKVFSREELELVASLCQQHDVVCITDEVYQWMVYDGHQHISIASLPGMWERTLTIGSAGKTFSATGWKVGWVLGPDHIMKHLRTVHQNSVFHCPTQSQAAVAESFEREQLLFRQPSSYFVQFPQAMQRCRDHMIHSLQSVGLKPIIPQGSYFLITDISDFKRKMPDLPGAVDEPYDRRFVKWMIKNKGLVAIPVSIFYSVPHQKHFDHYIRFCFVKDEATLQAMDEKLRKWKVEL

SEQ ID NO: 8 - protein, 422 aa, Macaca mulatta
MAKQLQARRLDGIDHNPWVEFVKLASEHDVVNLGQGFPDFPPPDFAVEAFQHAVSGDFMLNQYTKAFGYPPLTKVLASFFGKLLGQEMDPLRNVLVTVGGYGALFTAFQALVDEGDEVIIIEPFFDCYEPMTVMAGGRPVFVPLKPGPIQNGELGSSSNWQLDSMELASKFTSRTKALVLNTPNNPLGKVFSREELELVASLCQQHDVVCITDEVYQWMVYDGHPHISIASLPGMWERTLTIGSAGKTFSATGWKVGWVLGPDHIMKHLRTVHQNSIFHCPTQSQAAVAESFEREQLLFGQPSSYFVQFPQAMQRCRDHMVRSLQSVGLKPIVPQGSYFLITDISDFKRKMPDLPGAVDEPYDRRFVKWMIKNKGLVAIPVSIFCSVPHQKHFDHYIRFCFVKDEATLQAMDEKLRKWKAEL

SEQ ID NO: 9 - protein, 425 aa, Bos taurus
MAKRLQARRLDGIDHNPWVEFVQLASEEADVVNLGQGFPDFSPPEFAVEAFQHAVSGDFMLNQYTKAFGYPPLTKILANFFGKLLGQEIDPLKNVLVTVGAYGALFTAFQALVDEGDEVIIIEPFFDCYEPMTLMAGGRPVFVSLKPSPTQKGEPDSSSNWQLDPTELASKFTSRTKAFILNTPNNPLGKVFSKEELELVASLCQQHDVVCISDEVYQWMVFDGFQHISIASLPGMWERTLTIGSAGKTFSVTGWKVGWVLGPDSLMKHLRTVHQNSIYHCATQGQAAVAQSFEREQLHFGRPSSYFVQLPQYIQRCRDHMIQSLQSMGFRPVIPQGSYFLITDISDFKNKMPDLPGAAGEPYDRRFVKWMIKNKGLVAVPVSIFFSLPHQKFFDHYIRFCFVKDESTLRAMDQKLQKWKAELTP

SEQ ID NO: 10 - protein, 425 aa, Homo sapiens
MNYARFITAASAARNPSPIRTMTDILSRGPKSMISLAGGLPNPNMFPFKTAVITVENGKTIQFGEEMMKRALQYSPSAGIPELLSWLKQLQIKLHNPPTIHYPPSQGQMDLCVTSGSQQGLCKVFEMIINPGDNVLLDEPAYSGTLQSLHPLGCNIINVASDESGIVPDSLRDILSRWKPEDAKNPQKNTPKFLYTVPNGNNPTGNSLTSERKKEIYELARKYDFLIIEDDPYYFLQFNKFRVPTFLSMDVDGRVIRADSFSKIISSGLRIGFLTGPKPLIERVILHIQVSTLHPSTFNQLMISQLLHEWGEEGFMAHVDRVIDFYSNQKDAILAAADKWLTGLAEWHVPAAGMFLWIKVKGINDVKELIEEKAVKMGVLMLPGNAFYVDSSAPSPYLRASFSSASPEQMDVAFQVLAQLIKESL

SEQ ID NO: 11 - protein, 429 aa, Homo sapiens
MNYARFITAASAARNPSPIRTMSEKRADILSRGPKSMISLAGGLPNPNMFPFKTAVITVENGKTIQFGEEMMKRALQYSPSAGIPELLSWLKQLQIKLHNPPTIHYPPSQGQMDLCVTSGSQQGLCKVFEMIINPGDNVLLDEPAYSGTLQSLHPLGCNIINVASDESGIVPDSLRDILSRWKPEDAKNPQKNTPKFLYTVPNGNNPTGNSLTSERKKEIYELARKYDFLIIEDDPYYFLQFNKFRVPTFLSMDVDGRVIRADSFSKIISSGLRIGFLTGPKPLIERVILHIQVSTLHPSTFNQLMISQLLHEWGEEGFMAHVDRVIDFYSNQKDAILAAADKWLTGLAEWHVPAAGMFLWIKVKGINDVKELIEEKAVKMGVLMLPGNAFYVDSSAPSPYLRASFSSASPEQMDVAFQVLAQLIKESL

SEQ ID NO: 12 - protein, 425 aa, Rattus norvegicus
MNYSRFLTATSLARKTSPIRATVEIMSRAPKDIISLAPGSPNPKVFPFKSAVFTVENGSTIRFEGEMFQRALQYSSSYGIPELLSWLKQLQIKLHNPPTVNYSPNEGQMDLCITSGCQDGLCKVFEMLINPGDTVLVNEPLYSGALFAMKPLGCNFISVPSDDCGIIPEGLKKVLSQWKPEDSKDPTKRTPKFLYTIPNGNNPTGNSLTGDRKKEIYELARKYDFLIIEDDPYYFLQFTKPWEPTFLSMDVDGRVIRADSLSKVISSGLRVGFITGPKSLIQRIVLHTQISSLHPCTLSQLMISELLYQWGEEGFLAHVDRAIDFYKNQRDFILAAADKWLRGLAEWHVPKAGMFLWIKVNGISDAKKLIEEKAIEREILLVPGNSFFVDNSAPSSFFRASFSQVTPAQMDLVFQRLAQLIKDVS

SEQ ID NO: 13 - protein, 425 aa, Mus musculus
MNYSRFLTATSLARKPSPIRTTADILSKAPKTLISLAPGSPNPSMFPFKSAAFTVENGSTIRFEDDLIKRALQYSPSYGIPELLSWLKQFQVKLHNPPTVNYPPNQGQMDLCITSGCQDGLCKAFEMLINPGDTILVNEPLFPGTLYAMKPLGCNIINVPSDEHGIIPEGLKKILSQWKPEDSKDPTKKTPKFLYTVPNGNNPTGNSLTGDRKKEIYELARKYDFLIIEDDPYYFLQFSKPWEPTFLSMDVDGRVIRADTFSKTVSSGLRVGFMTGPKTLIQNIVLHTQVSSVHACTLSQLMILQLLHQWGEEGFLAHIDRTIDFYKNQRDSILAAADKWLRGLAEWHVPKAGMFLWIKVKGISDTKQLIEEKAIEREVLLVPGNGFFIDGSAPTSFFRASFSLATPAQMDTAFQRLAQLIKESL

SEQ ID NO: 14 - protein, 425 aa, Pan troglodytes
MNYARFITAASAARNPSPIRTMTDILSRGPKSMISLAGGLPNPNMFPFKTAVITVENGKTIQFGEEMMKRALQYSPSAGIPELLSWLKQLQIKLHNPPTIHYPPSQGQMDLCVTSGSQQGLCKVFEMIINPGDNVLLDEPAYAGTLQSLHPLGCNIINVASDESGIVPDSLRDILSRWKPEDSKNPQKNTPKFLYTVPNGNNPTGNSLTSERKKEIYELARKYDFLIIEDDPYYFLQFNKFRVPTFLSMDVDGRVIRADSFSKIISSGLRIGFLTGPKPLIERIILHIQVSTLHPSTFNQLMISQLLHEWGEEGFMAHVDRVIDFYSNQKDAILAAADKWLTGLAEWHVPAAGMFLWIKVKGINDVKELIEEKAVKMGVLMLPGNAFYVDSSAPSPYLRASFSSASPEQMDVAFQVLAQLIKESL

SEQ ID NO: 15 - protein, 425 aa, Macaca mulatta
MNYARFITAASAARNPSPIRTATEISSRGPKSMISLAGGLPNPNMFPFKTAVITVENGKTIEFGEEMMKRALQYSPSAGIPELLSWLKQLQIKLHNPPTVHYPPSQGQMDLCVTSGSQQGLCKVFEMIINPGDNVLLDEPAYSGTLQSLHPLGCNIINVASDEHGIVPDSLRDILSRWKPEDSKNPQKNTPKFLYTVPSGNNPTGNSLTSERKKEIYELARKYDFLIIEDDPYYFLQFNKFRVPTFLSMDVDGRVIRADSFSKIISSGLRIGFLTGPKPLIERVILHIQVSTLHPSTFNQLMISQLLHDWGEEGFMAHVDRVTDFYSNQKDAILAAADKWLTGLAEWHVPAAGMFLWIKVKGINDVKELIEEKAVKMGVLMLPGNAFYIDSSAPSPYLRASFSSASPEQMDMAFQVLAQLIKESL

SEQ ID NO: 16 - protein, 425 aa, Bos taurus
MNYARFITATSAARKPSTIRVMTEILSKAPKSVISLATGAPNPNTFPFKTAVITIENGKPIQFNEQMMKRALQYSQSAGIPELLSWLKQLQVKLHNPPTIHYAPTQGQMDLCVTCGSQEGLCKVFEMIVNPGDNILVNEPIYSGTIHALQPLGCNMINVSSDEHGIIPDSLREILSKWKPEDSKNPKKNSPKFLYTVPNGNNPSGNSLTAERKREIYELARKYDFLIIEDDPYYFMQFNKPWAPTFLSMDEDGRVIRADSFSKVLSSGLRIGFITGPKPLIERIVLHIQVSTMHPSTFAQLLVSQLLYQWGEEGFLGHVDRVIDFYRKQRDALMAAADKWLSGLAEWHVPTAGMFLWVKIKGIHDVRKLIEEKAFKKEIFMLPGCGFYTDSSAPCPYFRASFSSASPEQMDLAFQRLAQLIKESL

SEQ ID NO: 17 - protein, 454 aa, Homo sapiens
MFLAQRSLCSLSGRAKFLKTISSSKILGFSTSAKMSLKFTNAKRIEGLDSNVWIEFTKLAADPSVVNLGQGFPDISPPTYVKEELSKIAAIDSLNQYTRGFGHPSLVKALSYLYEKLYQKQIDSNKEILVTVGAYGSLFNTIQALIDEGDEVILIVPFYDCYEPMVRMAGATPVFIPLRSKPVYGKRWSSSDWTLDPQELESKFNSKTKAIILNTPHNPLGKVYNREELQVIADLCIKYDTLCISDEVYEWLVYSGNKHLKIATFPGMWERTITIGSAGKTFSVTGWKLGWSIGPNHLIKHLQTVQQNTIYTCATPLQEALAQAFWIDIKRMDDPECYFNSLPKELEVKRDRMVRLLESVGLKPIVPDGGYFIIADVSLLDPDLSDMKNNEPYDYKFVKWMTKHKKLSAIPVSAFCNSETKSQFEKFVRFCFIKKDSTLDAAEEIIKAWSVQKS

SEQ ID NO: 18 - protein, 167 aa, Homo sapiens
MFLAQRSLCSLSGRAKFLKTISSSKILGFSTSAKMSLKFTNAKRIEGLDSNVWIEFTKLAADPSVVNLGQGFPDISPPTYVKEELSKIAAIDSLNQYTRGFGHPSLVKALSYLYEKLYQKQIDSNKEILVTVGAYGSLFNTIQALIDEGDEYNACTVKFTNLKCTAG

SEQ ID NO: 19 - protein, 420 aa, Homo sapiens
MSLKFTNAKRIEGLDSNVWIEFTKLAADPSVVNLGQGFPDISPPTYVKEELSKIAAIDSLNQYTRGFGHPSLVKALSYLYEKLYQKQIDSNKEILVTVGAYGSLFNTIQALIDEGDEVILIVPFYDCYEPMVRMAGATPVFIPLRSKPVYGKRWSSSDWTLDPQELESKFNSKTKAIILNTPHNPLGKVYNREELQVIADLCIKYDTLCISDEVYEWLVYSGNKHLKIATFPGMWERTITIGSAGKTFSVTGWKLGWSIGPNHLIKHLQTVQQNTIYTCATPLQEALAQAFWIDIKRMDDPECYFNSLPKELEVKRDRMVRLLESVGLKPIVPDGGYFIIADVSLLDPDLSDMKNNEPYDYKFVKWMTKHKKLSAIPVSAFCNSETKSQFEKFVRFCFIKKDSTLDAAEEIIKAWSVQKS

SEQ ID NO: 20 - protein, 454 aa, Rattus norvegicus
MLLAQRRLFSLGCRAKPIKTIYSSKVLGLSTSAKMALRFKNAKRIEGLDQNVWVEFTKLAADPSVVNLGQGFPDITLPSYVQEELSKAAFIDNLNQYTRGFGHPSLVKALSCLYGKIYQKQIDPNEEILVTVGGYGSLFNAIQGLVDPGDEVIIMVPFYDCYEPMVKMAGAVPVFIPLRSKRTDGMKWTSSDWTFNPQELESKFSSKTKAIILNTPHNPIGKVYTREELQVIADLCIKHDTLCISDEVYEWLVYTGHKHIKVASLPGMWDRTLTIGSAGKTFSVTGWKLGWSIGPGHLIKHLRTVQQTSVYTCATPLQAALAEAFWIDIKRMDDPECYFNSLPKELEVKRDRMACLLNSVGLKPIIPDGGYFIIADVSSLGVDLSDVKSDEPYDYKFVKWMTKNKKLSAIPVSAFCDSESKPHFEKLVRFCFIKKDSTLDAAEEIFRTWNSRKS

SEQ ID NO: 21 - protein, 455 aa, Mus musculus
MLLAQRRLISLGCRSKPIKTIYSSSKVLGLCTSAKMALKFKNAKRIEGLDSNVWVEFTKLAADPSVVNLGQGFPDISPPSYVKEELSKAAFIDNMNQYTRGFGHPALVKALSCLYGKIYQRQIDPNEEILVAVGAYGSLFNSIQGLVDPGDEVIIMVPFYDCYEPMVRMAGAVPVFIPLRSKPTDGMKWTSSDWTFDPRELESKFSSKTKAIILNTPHNPLGKVYTRQELQVIADLCVKHDTLCISDEVYEWLVYTGHTHVKIATLPGMWERTITIGSAGKTFSVTGWKLGWSIGPAHLIKHLQTVQQNSFYTCATPLQAALAEAFWIDIKRMDDPECYFNSLPKELEVKRDRMVRLLNSVGLKPIVPDGGYFIIADVSSLGADLSDMNSDEPYDYKFVKWMTKHKKLTAIPVSAFCDSKSKPHFEKLVRFCFIKKDSTLDAAEEIFRAWNSQKS

SEQ ID NO: 22 - protein, 420 aa, Mus musculus
MALKFKNAKRIEGLDSNVWVEFTKLAADPSVVNLGQGFPDISPPSYVKEELSKAAFIDNMNQYTRGFGHPALVKALSCLYGKIYQRQIDPNEEILVAVGAYGSLFNSIQGLVDPGDEVIIMVPFYDCYEPMVRMAGAVPVFIPLRSKPTDGMKWTSSDWTFDPRELESKFSSKTKAIILNTPHNPLGKVYTRQELQVIADLCVKHDTLCISDEVYEWLVYTGHTHVKIATLPGMWERTITIGSAGKTFSVTGWKLGWSIGPAHLIKHLQTVQQNSFYTCATPLQAALAEAFWIDIKRMDDPECYFNSLPKELEVKRDRMVRLLNSVGLKPIVPDGGYFIIADVSSLGADLSDMNSDEPYDYKFVKWMTKHKKLTAIPVSAFCDSKSKPHFEKLVRFCFIKKDSTLDAAEEIFRAWNSQKS

SEQ ID NO: 23 - protein, 454 aa, Pan troglodytes
MFLAQRSLCSLSGTAKFLKTISSSKIFGFSTSAKMSLKFTNAKRIEGLDSNVWIEFTKLAADPSVVNLGQGFPDISPPTYVKEELSKIAAIDSLNQYTRGFGHPSLVKALSCLYEKLYQKQIDSNKEILVTVGAYGSLFNTIQALIDEGDEVILIVPFYDCYEPMVRMAGATPVFIPLRSKPVYGKRWSSSDWTLDPQELESKFNSKTKAIILNTPHNPLGKVYNKEELQVISDLCIKYDTLCISDEVYEWLVYSGNKHLKIATFPGMWERTITIGSAGKTFSVTGWKLGWSIGPNHLIKHLQTVQQNTIYTCATPLQEALAQAFWIDIKRMDDPECYFNSLPKELEVKRDRMVRLLESVGLKPIVPDGGYFIIADVSLLDPDLSDMKNNEPYDYKFVKWMTKHKKLSAIPVSAFCNSETKSQFEKFVRFCFIKKDSTLDAAEEIIKAWSVQKS

SEQ ID NO: 24 - protein, 454 aa, Macaca mulatta
MFLAQRSLCFPSGRAKFLKTISSSKILGFSASAKMSLKFTNAKRIEGLDGNMWIEFTKLAADPSVVNLGQGFPDISPPTYVKEELSKISAIDSLNQYTRGFGHPSLVKALSYLYEKLYQKQIDSNKEILVTVGAYGSLFNTVQALIDEGDEVILIVPFYDCYEPMVRMAGATPVFIPLRSKPVDGKRWSSSDWTLDPQELESKFNSKTKAIILNTPHNPLGKVYNKEELQVIADLCIKYDTLCISDEVYEWLVYSGNKHLKIATFPGMWERTITIGSAGKTFSVTGWKLGWSIGPNHLIKHLQTVQQNTIYTCATPLQEALAQAFWIDIKRMDDPECYFNSLPKELEVKRDRMVHLLESVGLKPIVPDGGYFIIADVSLLDPDLSDMKNNEPYDYKFVKWMTKHKKLSAIPVSAFCNSETKSQFEKFVRFCFIKKDSTLDAAEEIIKAWSVQKS

SEQ ID NO: 25 - protein, 455 aa, Bos taurus
MFLAWERLCTLSCRPKFLKTVWASKILGLSTSAKMSLRFKNAKRIEGLDSNIWIEFTKLAADPSVVNLGQGLPDISPPVYVKEELSKIAAIDNLNQYTRGFGHPSLVKALSCLYEKFYHNKINPNEEILVTVGAYGSLFNAIQGLIDEGDEVIVIVPFFDCYESMVRMAGATPVFVPLRCKPVDGKKCSSSDWTLDPQELASKFNSKTKAIILNTPHNPLGKVYTKEELQVIADLCIKYDTLCISDEVYEWLVYTGNKHFKIATFPGMWERTITIGSAGKTFSVTGWKLGWSIGPKHLIKHLQTVQQNTVYTCATPLQEALAQAFWIDIKRMDDPECYFNSLPKELEVKRDRMVHLLESVGLKSIVPDGGYFIIADVSLLDVDLLDMKDSNEPYDYKFVKWMIKNKKLSAIPVSAFCNAETKSQFEKFVRFCFIKKDSTLDAAEEIIKAWSRQNS

SEQ ID NO: 26 - protein, 430 aa, Homo sapiens
MALLHSGRVLPGIAAAFHPGLAAAASARASSWWTHVEMGPPDPILGVTEAFKRDTNSKKMNLGVGAYRDDNGKPYVLPSVRKAEAQIAAKNLDKEYLPIGGLAEFCKASAELALGENSEVLKSGRFVTVQTISGTGALRIGASFLQRFFKFSRDVFLPKPTWGNHTPIFRDAGMQLQGYRYYDPKTCGFDFTGAVEDISKIPEQSVLLLHACAHNPTGVDPRPEQWKEIATVVKKRNLFAFFDMAYQGFASGDGDKDAWAVRHFIEQGINVCLCQSYAKNMGLYGERVGAFTMVCKDADEAKRVESQLKILIRPMYSNPPLNGARIAAAILNTPDLRKQWLQEVKVMADRIIGMRTQLVSNLKKEGSTHNWQHITDQIGMFCFTGLKPEQVERLIKEFSIYMTKDGRISVAGVTSSNVGYLAHAIHQVTK

SEQ ID NO: 27 - protein, 387 aa, Homo sapiens
MALLHSGRVLPGIAAAFHPGLAAAASARASSWWTHVEMGPPDPILGVTEAFKRDTNSKKMNLGVGAYRDDNGKPYVLPSVRKFVTVQTISGTGALRIGASFLQRFFKFSRDVFLPKPTWGNHTPIFRDAGMQLQGYRYYDPKTCGFDFTGAVEDISKIPEQSVLLLHACAHNPTGVDPRPEQWKEIATVVKKRNLFAFFDMAYQGFASGDGDKDAWAVRHFIEQGINVCLCQSYAKNMGLYGERVGAFTMVCKDADEAKRVESQLKILIRPMYSNPPLNGARIAAAILNTPDLRKQWLQEVKVMADRIIGMRTQLVSNLKKEGSTHNWQHITDQIGMFCFTGLKPEQVERLIKEFSIYMTKDGRISVAGVTSSNVGYLAHAIHQVTK

SEQ ID NO: 28 - protein, 430 aa, Rattus norvegicus
MALLHSGRVLSGMAAAFHPGLAAAASARASSWWTHVEMGPPDPILGVTEAFKRDTNSKKMNLGVGAYRDDNGKPYVLPSVRKAEAQIAGKNLDKEYLPIGGLADFCKASAELALGENSEVLKSGRFVTVQTISGTGALRVGASFLQRFFKFSRDVFLPKPSWGNHTPIFRDAGMQLQGYRYYDPKTCGFDFSGALEDISKIPEQSVLLLHACAHNPTGVDPRPEQWKEMAAVVKKKNLFAFFDMAYQGFASGDGDKDAWAVRHFIEQGINVCLCQSYAKNMGLYGERVGAFTVVCKDAEEAKRVESQLKILIRPLYSNPPLNGARIAATILTSPDLRKQWLQEVKGMADRIISMRTQLVSNLKKEGSSHNWQHITDQIGMFCFTGLKPEQVERLTKEFSVYMTKDGRISVAGVTSGNVGYLAHAIHQVTK

SEQ ID NO: 29 - protein, 430 aa, Mus musculus
MALLHSSRILSGMAAAFHPGLAAAASARASSWWTHVEMGPPDPILGVTEAFKRDTNSKKMNLGVGAYRDDNGKPYVLPSVRKAEAQIAAKNLDKEYLPIGGLAEFCKASAELALGENNEVLKSGRFVTVQTISGTGALRVGASFLQRFFKFSRDVFLPKPSWGNHTPIFRDAGMQLQGYRYYDPKTCGFDFSGALEDISKIPEQSVLLLHACAHNPTGVDPRPEQWKEIASVVKKKNLFAFFDMAYQGFASGDGDKDAWAVRHFIEQGINVCLCQSYAKNMGLYGERVGAFTVVCKDAEEAKRVESQLKILIRPLYSNPPLNGARIAATILTSPDLRKQWLQEVKGMADRIISMRTQLVSNLKKEGSSHNWQHITDQIGMFCFTGLKPEQVERLTKEFSVYMTKDGRISVAGVTSGNVGYLAHAIHQVTK

SEQ ID NO: 30 - protein, 430 aa, Pan troglodytes
MALLHSGRVLPGIAAAFHPGLAAAASARASSWWTHVEMGPPDPILGVTEAFKRDTNSKKMNLGVGAYRDDNGKPYVLPSVRKAEAQIAAKNLDKEYLPIGGLAEFCKASAELALGENSEVLKSGRFVTVQTISGTGALRIGASFLQRFFKFSRDVFLPKPTWGNHTPIFRDAGMQLQGYRYYDPKTCGFDFTGAVEDISKIPEQSVLLLHACAHNPTGVDPRPEQWKEIATVVKKRNLFAFFDMAYQGFASGDGDKDAWAVRHFIEQGINVCLCQSYAKNMGLYGERVGAFTMVCKDADEAKRVESQLKILIRPMYSNPPLNGARIAAAILNTPDLRKQWLQEVKGMADRIIGMRTQLVSNLKKEGSTHNWQHITDQIGMFCFTGLKPEQVERLIKEFSIYMTKDGRISVAGVTSSNVGYLAHAIHQVTK

SEQ ID NO: 31 - protein, 430 aa, Macaca mulatta
MALLHSGRVLSGIAAAFHPGLAAAASARASSWWTHVEMGPPDPILGVTEAFKRDTNSKKMNLGVGAYRDDNGKPYVLPSVRKAEAQIAAKNLDKEYLPIGGLAEFCKASAELALGENSEVLKSGRFVTVQTISGTGALRIGASFLQRFFKFSRDVFLPKPSWGNHTPIFRDAGMQLQGYRYYDPKTCGFDFTGAVEDISKIPEQSVLLLHACAHNPTGVDPRPEQWKEIATVVKKRNLFAFFDMAYQGFASGDGDKDAWAVRHFIEQGINVCLCQSYAKNMGLYGERVGAFTMVCKDADEAKRVESQLKILIRPMYSNPPLNGARIAAAILNTPDLRKQWLQEVKGMADRIIGMRTQLVSNLKKEGSIHNWQHITDQIGMFCFTGLKPEQVERLTKEFSIYMTKDGRISVAGVTSGNVGYLAHAIHQVTK

SEQ ID NO: 32 - protein, 430 aa, Bos taurus
MALLHSGRFLSGVAAAFHPGLAAAASARASSWWAHVEMGPPDPILGVTEAFKRDTNSKKMNLGVGAYRDDNGKPYVLPSVRKAEAQIAAKNLDKEYLPIAGLAEFCKASAELALGENNEVLKSGRYVTVQTISGTGALRIGASFLQRFFKFSRDVFLPKPTWGNHTPIFRDAGMQLQSYRYYDPKTCGFDFTGAIEDISKIPAQSVILLHACAHNPTGVDPRPEQWKEMATVVKKNNLFAFFDMAYQGFASGDGNKDAWAVRHFIEQGINVCLCQSYAKNMGLYGERVGAFTVVCKDAEEAKRVESQLKILIRPMYSNPPINGARIASTILTSPDLRKQWLHEVKGMADRIISMRTQLVSNLKKEGSSHNWQHIIDQIGMFCYTGLKPEQVERLTKEFSIYMTKDGRISVAGVTSGNVAYLAHAIHQVTK